European Patent Application EP 4 414 454 A1, published August 14, 2024. Title: Modified Transglutaminase. Applicant: Amano Enzyme Inc. The sequence listing filed with the application follows.

SEQUENCE LISTING (3 sequences)

SEQ ID NO: 1 - protein, 331 aa, S2P/S23Y/Y24N/H289Y/K294L mutation of transglutaminase derived from Streptomyces mobaraensis
  REGION 1..331: note = S2P/S23Y/Y24N/H289Y/K294L mutation of transglutaminase derivedfrom Streptomyces mobaraensis
DPDDRVTPPAEPLDRMPDPYRPYNGRAETVVNNYIRKWQQVYSHRDGRKQQMTEEQREWLSYGCVGVTWVNSGQYPTNRLAFASFDEDRFKNELKNGRPRSGETRAEFEGRVAKESFDEEKGFQRAREVASVMNRALENAHDESAYLDNLKKELANGNDALRNEDARSPFYSALRNTPSFKERNGGNHDPSRMKAVIYSKHFWSGQDRSSSADKRKYGDPDAFRPAPGTGLVDMSRDRNIPRSPTSPGEGFVNFDYGWFGAQTEADADKTVWTHGNHYHAPNGSLGAMYVYESLFRNWSEGYSDFDRGAYVITFIPKSWNTAPDKVKQGWP

SEQ ID NO: 2 - protein, 331 aa, Streptomyces mobaraensis
DSDDRVTPPAEPLDRMPDPYRPSYGRAETVVNNYIRKWQQVYSHRDGRKQQMTEEQREWLSYGCVGVTWVNSGQYPTNRLAFASFDEDRFKNELKNGRPRSGETRAEFEGRVAKESFDEEKGFQRAREVASVMNRALENAHDESAYLDNLKKELANGNDALRNEDARSPFYSALRNTPSFKERNGGNHDPSRMKAVIYSKHFWSGQDRSSSADKRKYGDPDAFRPAPGTGLVDMSRDRNIPRSPTSPGEGFVNFDYGWFGAQTEADADKTVWTHGNHYHAPNGSLGAMHVYESKFRNWSEGYSDFDRGAYVITFIPKSWNTAPDKVKQGWP

SEQ ID NO: 3 - DNA, 996 bp, synthetic construct
  misc_feature 1..996: note = base sequence coding S2P/S23Y/Y24N/H289Y/K294L mutation oftransglutaminase derived from Streptomyces mobaraensis
  source 1..996: mol_type = other DNA
gacccggacgacagggtcacccctcccgccgagccgctcgacaggatgcccgacccgtaccgtccctataacggcagggccgagacggtcgtcaacaactacatacgcaagtggcagcaggtctacagccaccgcgacggcaggaagcagcagatgaccgaggagcagcgggagtggctgtcctacggctgcgtcggtgtcacctgggtcaattcgggtcagtacccgacgaacagactggccttcgcgtccttcgacgaggacaggttcaagaacgagctgaagaacggcaggccccggtccggcgagacgcgggcggagttcgagggccgcgtcgcgaaggagagcttcgacgaggagaagggcttccagcgggcgcgtgaggtggcgtccgtcatgaacagggccctggagaacgcccacgacgagagcgcttacctcgacaacctcaagaaggaactggcgaacggcaacgacgccctgcgcaacgaggacgcccgttccccgttctactcggcgctgcggaacacgccgtccttcaaggagcggaacggaggcaatcacgacccgtccaggatgaaggccgtcatctactcgaagcacttctggagcggccaggaccggtcgagttcggccgacaagaggaagtacggcgacccggacgccttccgccccgccccgggcaccggcctggtcgacatgtcgagggacaggaacattccgcgcagccccaccagccccggtgagggattcgtcaatttcgactacggctggttcggcgcccagacggaagcggacgccgacaagaccgtctggacccacggaaatcactatcacgcgcccaatggcagcctgggtgccatgtatgtctacgagagcctgttccgcaactggtccgagggttactcggacttcgaccgcggagcctatgtgatcaccttcatccccaagagctggaacaccgcccccgacaaggtaaagcagggctggccgtga